European Patent Specification EP 3 302 557 B1, published January 31, 2024. Title: ENHANCING THE THERAPEUTIC ACTIVITY OF AN IMMUNE CHECKPOINT INHIBITOR. Applicant: Maine Medical Center Research Institute. The sequence listing filed with the application follows.

SEQUENCE LISTING (15 sequences)

SEQ ID NO: 1 - protein, 6 aa, Artificial Sequence
  Synthetic peptide
RGDKGE

SEQ ID NO: 2 - protein, 9 aa, Artificial Sequence
  Synthetic peptide
KGDRGDAPG

SEQ ID NO: 3 - protein, 9 aa, Artificial Sequence
  Synthetic peptide
QGPRGDKGE

SEQ ID NO: 4 - protein, 9 aa, Artificial Sequence
  Synthetic peptide
QGPSGSPGE

SEQ ID NO: 5 - protein, 11 aa, Artificial Sequence
  Synthetic peptide
CKGDRGDAPGC

SEQ ID NO: 6 - protein, 11 aa, Artificial Sequence
  Synthetic peptide
CQGPRGDKGEC

SEQ ID NO: 7 - protein, 11 aa, Artificial Sequence
  Synthetic peptide
CAGSRGDGGPC

SEQ ID NO: 8 - protein, 10 aa, Artificial Sequence
  Synthetic peptide
CQGIRGDKGE

SEQ ID NO: 9 - protein, 11 aa, Artificial Sequence
  Synthetic peptide
CRGPRGDQGPC

SEQ ID NO: 10 - protein, 11 aa, Artificial Sequence
  Synthetic peptide
CQGPSGAPGEC

SEQ ID NO: 11 - protein, 6 aa, Artificial Sequence
  Synthetic peptide
RGDAPG

SEQ ID NO: 12 - protein, 9 aa, Artificial Sequence
  Synthetic peptide
AGSRGDGGP

SEQ ID NO: 13 - protein, 9 aa, Artificial Sequence
  Synthetic peptide
QGIRGDKGE

SEQ ID NO: 14 - protein, 9 aa, Artificial Sequence
  Synthetic peptide
RGPRGDQGP

SEQ ID NO: 15 - protein, 9 aa, Artificial Sequence
  Synthetic peptide
QGPSGAPGE